European Patent Application EP 4 241 776 A1, published September 13, 2023. Title: PHARMACEUTICAL COMPOSITION FOR PREVENTING OR TREATING FIBROSIS COMPRISING ISOLATED MITOCHONDRIA. Applicant: Paean Biotechnology Inc. The sequence listing filed with the application follows.

SEQUENCE LISTING (10 sequences)

SEQ ID NO: 1 - DNA, 19 bp, Artificial Sequence
  CTGF-S
ggcttaccgactggaagac

SEQ ID NO: 2 - DNA, 18 bp, Artificial Sequence
  CTGF-AS
aggaggcgttgtcattgg

SEQ ID NO: 3 - DNA, 20 bp, Artificial Sequence
  Fibronectin-S
gtggctgaagacacaaggaa

SEQ ID NO: 4 - DNA, 19 bp, Artificial Sequence
  Fibronectin-AS
cctgccattgtaggtgaat

SEQ ID NO: 5 - DNA, 20 bp, Artificial Sequence
  NOX4-S
cacctctgcctgttcatctg

SEQ ID NO: 6 - DNA, 21 bp, Artificial Sequence
  NOX4-AS
ggctctgcttagacacaatcc

SEQ ID NO: 7 - DNA, 22 bp, Artificial Sequence
  Alpha-SMA-S
gcccagccaagcactgtcagga

SEQ ID NO: 8 - DNA, 23 bp, Artificial Sequence
  Alpha-SMA-AS
tcccaccatcaccccctgatgtc

SEQ ID NO: 9 - DNA, 22 bp, Artificial Sequence
  GAPDH-S
gtctcctctgacttcaacagcg

SEQ ID NO: 10 - DNA, 22 bp, Artificial Sequence
  GAPDH-AS
accaccctgttgctgtagccaa